European Patent Application EP 4 644 427 A2, published November 5, 2025. Title: MANAbodies AND METHODS OF USING. Applicant: The Johns Hopkins University. Application EP. The sequence listing filed with the application follows.

SEQUENCE LISTING (420 sequences)

SEQ ID NO: 1 - protein, 10 aa, synthetic construct
SPNGTIQNIL

SEQ ID NO: 2 - protein, 10 aa, synthetic construct
SPNGTIRNIL

SEQ ID NO: 3 - protein, 243 aa, synthetic construct
DIQMTQSPSSLSASVGDRVTITCRASQDVNTAVAWYQQKPGKAPKLLIYSASFLYSGVPSRFSGSRSGTDFTLTISSLQPEDFATYYCQQYSYSPPTFGQGTKVEIKRTGGGSGGGGSGGGASEVQLVESGGGLVQPGGSLRLSCAASGFNISDTYIHWVRQAPGKGLEWVASISPRTGYNRYADSVKGRFTISADTSKNTAYLQMNSLRAEDTAVYYCSRAYYSYAYAMDVWGQGTLVTVSS

SEQ ID NO: 4 - protein, 242 aa, synthetic construct
DIQMTQSPSSLSASVGDRVTITCRASQDVNTAVAWYQQKPGKAPKLLIYSASFLYSGVPSRFSGSRSGTDFTLTISSLQPEDFATYYCQQGKAYWPATFGQGTKVEIKRTGGGSGGGGSGGGASEVQLVESGGGLVQPGGSLRLSCAASGFNVGHYRMHWVRQAPGKGLEWVAMVSPNGYYTYYADSVKGRFTISADTSKNTAYLQMNSLRAEDTAVYYCSRGYSSYAFDYWGQGTLVTVSS

SEQ ID NO: 5 - protein, 241 aa, synthetic construct
DIQMTQSPSSLSASVGDRVTITCRASQDVNTAVAWYQQKPGKAPKLLIYSASFLYSGVPSRFSGSRSGTDFTLTISSLQPEDFATYYCQQVYSSPFTFGQGTKVEIKRTGGGSGGGGSGGGASEVQLVESGGGLVQPGGSLRLSCAASGFNVKYYMMHWVRQAPGKGLEWVAAISPGYDYTYYADSVKGRFTISADTSKNTAYLQMNSLRAEDTAVYYCSRSYWRYSVDVWGQGTLVTVSS

SEQ ID NO: 6 - protein, 245 aa, synthetic construct
DIQMTQSPSSLSASVGDRVTITCRASQDVNTAVAWYQQKPGKAPKLLIYSASFLYSGVPSRFSGSRSGTDFTLTISSLQPEDFATYYCQQYSLYSPMTFGQGTKVEIKRTGGGSGGGGSGGGASEVQLVESGGGLVQPGGSLRLSCAASGFNSFLSIHWVRQAPGKGLEWVAHIFPSSDYTSYADSVKGRFTISADTSKNTAYLQMNSLRAEDTAVYYCSRGKHSSDSNYYMDYWGQGTLVTVSS

SEQ ID NO: 7 - skipped

SEQ ID NO: 8 - protein, 241 aa, synthetic construct
DIQMTQSPSSLSASVGDRVTITCRASQDVNTAVAWYQQKPGKAPKLLIYSASFLYSGVPSRFSGSRSGTDFTLTISSLQPEDFATYYCQQSYYMPFTFGQGTKVEIKRTGGGSGGGGSGGGASEVQLVESGGGLVQPGGSLRLSCAASGFNIFRGYMHWVRQAPGKGLEWVAMISPHSDYTSYADSVKGRFTISADTSKNTAYLQMNSLRAEDTAVYYCSRSYGWAAFDYWGQGTLVTVSS

SEQ ID NO: 9 - protein, 10 aa, synthetic construct
RPIPIKYKAM

SEQ ID NO: 10 - protein, 10 aa, synthetic construct
KPITIGRHAH

SEQ ID NO: 11 - protein, 9 aa, synthetic construct
AVGVGKSAL

SEQ ID NO: 12 - protein, 9 aa, synthetic construct
AGGVGKSAL

SEQ ID NO: 13 - protein, 9 aa, synthetic construct
IMQLMPFGC

SEQ ID NO: 14 - protein, 9 aa, synthetic construct
ITQLMPFGC

SEQ ID NO: 15 - protein, 10 aa, synthetic construct
GMNQRPILTI

SEQ ID NO: 16 - protein, 10 aa, synthetic construct
GMNWRPILTI

SEQ ID NO: 17 - protein, 10 aa, synthetic construct
GMNRRPILTI

SEQ ID NO: 18 - protein, 9 aa, synthetic construct
LVVVGAVGV

SEQ ID NO: 19 - protein, 9 aa, synthetic construct
LVVVGAGGV

SEQ ID NO: 20 - protein, 10 aa, synthetic construct
VVVGACGVGK

SEQ ID NO: 21 - protein, 10 aa, synthetic construct
VVVGADGVGK

SEQ ID NO: 22 - protein, 9 aa, synthetic construct
VVGAVGVGK

SEQ ID NO: 23 - protein, 10 aa, synthetic construct
VVVGAGGVGK

SEQ ID NO: 24 - protein, 9 aa, synthetic construct
VVGADGVGK

SEQ ID NO: 25 - protein, 9 aa, synthetic construct
VVGAGGVGK

SEQ ID NO: 26 - protein, 9 aa, synthetic construct
TTAPFLSGK

SEQ ID NO: 27 - protein, 9 aa, synthetic construct
TTAPSLSGK

SEQ ID NO: 28 - protein, 10 aa, synthetic construct
ILDTAGHEEY

SEQ ID NO: 29 - protein, 10 aa, synthetic construct
ILDTAGQEEY

SEQ ID NO: 30 - protein, 10 aa, synthetic construct
ILDTAGKEEY

SEQ ID NO: 31 - protein, 10 aa, synthetic construct
ILDTAGLEEY

SEQ ID NO: 32 - protein, 10 aa, synthetic construct
ILDTAGREEY

SEQ ID NO: 33 - protein, 6 aa, synthetic construct
QDVNTA

SEQ ID NO: 34 - protein, 9 aa, synthetic construct
QQYDYAPIT

SEQ ID NO: 35 - protein, 11 aa, synthetic construct
QQSPYYYLPIT

SEQ ID NO: 36 - protein, 9 aa, synthetic construct
QQYYYSPVT

SEQ ID NO: 37 - protein, 9 aa, synthetic construct
QQHYGNPFT

SEQ ID NO: 38 - protein, 9 aa, synthetic construct
QQSYYSPPT

SEQ ID NO: 39 - protein, 9 aa, synthetic construct
QQYYSYPPT

SEQ ID NO: 40 - protein, 9 aa, synthetic construct
QQYYYYPPT

SEQ ID NO: 41 - protein, 8 aa, synthetic construct
GFNISWYQ

SEQ ID NO: 42 - protein, 8 aa, synthetic construct
GFNVSWSY

SEQ ID NO: 43 - protein, 8 aa, synthetic construct
GFNISWNQ

SEQ ID NO: 44 - protein, 8 aa, synthetic construct
GFNVGYYG

SEQ ID NO: 45 - protein, 8 aa, synthetic construct
GFNITSSY

SEQ ID NO: 46 - protein, 8 aa, synthetic construct
GFNINSSY

SEQ ID NO: 47 - protein, 8 aa, synthetic construct
GFNISTSY

SEQ ID NO: 48 - protein, 8 aa, synthetic construct
VTPYSGYT

SEQ ID NO: 49 - protein, 8 aa, synthetic construct
IYGDSGYT

SEQ ID NO: 50 - protein, 8 aa, synthetic construct
VSPYSGYT

SEQ ID NO: 51 - protein, 8 aa, synthetic construct
VSGMEGYT

SEQ ID NO: 52 - protein, 8 aa, synthetic construct
ISPADGYN

SEQ ID NO: 53 - protein, 8 aa, synthetic construct
ISPTDGYY

SEQ ID NO: 54 - protein, 8 aa, synthetic construct
IDPNDGYS

SEQ ID NO: 55 - protein, 10 aa, synthetic construct
SRSYTDGFDY

SEQ ID NO: 56 - protein, 14 aa, synthetic construct
SRGQWEASYYAMDY

SEQ ID NO: 57 - protein, 10 aa, synthetic construct
SRSDYYAMDY

SEQ ID NO: 58 - protein, 11 aa, synthetic construct
SRDIYGYAMDV

SEQ ID NO: 59 - protein, 13 aa, synthetic construct
SRTDSTAYTAMDV

SEQ ID NO: 60 - protein, 13 aa, synthetic construct
SRTSDTSYAAMDV

SEQ ID NO: 61 - protein, 13 aa, synthetic construct
SRTNNTAADAMDV

SEQ ID NO: 62 - protein, 9 aa, synthetic construct
QQYSYSPPT

SEQ ID NO: 63 - protein, 10 aa, synthetic construct
QQGKAYWPAT

SEQ ID NO: 64 - protein, 9 aa, synthetic construct
QQVYSSPFT

SEQ ID NO: 65 - protein, 10 aa, synthetic construct
QQYSLYSPMT

SEQ ID NO: 66 - protein, 9 aa, synthetic construct
QQSYYMPFT

SEQ ID NO: 67 - protein, 8 aa, synthetic construct
GFNISDTY

SEQ ID NO: 68 - protein, 8 aa, synthetic construct
GFNVGHYR

SEQ ID NO: 69 - protein, 8 aa, synthetic construct
GFNVKYYM

SEQ ID NO: 70 - protein, 7 aa, synthetic construct
GFNSFLS

SEQ ID NO: 71 - protein, 8 aa, synthetic construct
GFNIFRGY

SEQ ID NO: 72 - protein, 8 aa, synthetic construct
ISPRTGYN

SEQ ID NO: 73 - protein, 8 aa, synthetic construct
VSPNGYYT

SEQ ID NO: 74 - protein, 8 aa, synthetic construct
ISPGYDYT

SEQ ID NO: 75 - protein, 8 aa, synthetic construct
IFPSSDYT

SEQ ID NO: 76 - protein, 8 aa, synthetic construct
ISPHSDYT

SEQ ID NO: 77 - protein, 13 aa, synthetic construct
SRAYYSYAYAMDV

SEQ ID NO: 78 - protein, 11 aa, synthetic construct
SRGYSSYAFDY

SEQ ID NO: 79 - protein, 11 aa, synthetic construct
SRSYWRYSVDV

SEQ ID NO: 80 - protein, 15 aa, synthetic construct
SRGKHSSDSNYYMDY

SEQ ID NO: 81 - protein, 11 aa, synthetic construct
SRSYGWAAFDY

SEQ ID NO: 82 - protein, 9 aa, synthetic construct
QQSGYAPIT

SEQ ID NO: 83 - protein, 9 aa, synthetic construct
QQYSYAPIT

SEQ ID NO: 84 - protein, 9 aa, synthetic construct
QQSLYGPFT

SEQ ID NO: 85 - protein, 9 aa, synthetic construct
QQYSYSPIT

SEQ ID NO: 86 - protein, 9 aa, synthetic construct
QQSGYQPDT

SEQ ID NO: 87 - protein, 9 aa, synthetic construct
QQYLYQPWT

SEQ ID NO: 88 - protein, 9 aa, synthetic construct
QQGLYYPWT

SEQ ID NO: 89 - protein, 8 aa, synthetic construct
GFNISYYS

SEQ ID NO: 90 - protein, 8 aa, synthetic construct
GFNIGYYT

SEQ ID NO: 91 - protein, 8 aa, synthetic construct
GFNIAYEY

SEQ ID NO: 92 - protein, 8 aa, synthetic construct
GFNLFGYG

SEQ ID NO: 93 - protein, 8 aa, synthetic construct
GFNISWYA

SEQ ID NO: 94 - protein, 8 aa, synthetic construct
GFNIDYYG

SEQ ID NO: 95 - protein, 8 aa, synthetic construct
GFNVSYSS

SEQ ID NO: 96 - protein, 8 aa, synthetic construct
VDPDSDYT

SEQ ID NO: 97 - protein, 8 aa, synthetic construct
VSPWSYST

SEQ ID NO: 98 - protein, 8 aa, synthetic construct
IGPDSGYT

SEQ ID NO: 99 - protein, 8 aa, synthetic construct
IGPYYYYT

SEQ ID NO: 100 - protein, 8 aa, synthetic construct
IWPDSDWT

SEQ ID NO: 101 - protein, 8 aa, synthetic construct
LYGGSDST

SEQ ID NO: 102 - protein, 8 aa, synthetic construct
IWPDSGQT

SEQ ID NO: 103 - protein, 12 aa, synthetic construct
SRSWIHMFSMDY

SEQ ID NO: 104 - protein, 11 aa, synthetic construct
SRDHWDEAFDV

SEQ ID NO: 105 - protein, 13 aa, synthetic construct
SRVWYYSTYGMDY

SEQ ID NO: 106 - protein, 11 aa, synthetic construct
SRENYDMAMDY

SEQ ID NO: 107 - protein, 11 aa, synthetic construct
SRYYYSSAFDV

SEQ ID NO: 108 - protein, 10 aa, synthetic construct
SRQYSAYFDY

SEQ ID NO: 109 - protein, 11 aa, synthetic construct
SRSSYFDAMDY

SEQ ID NO: 110 - protein, 9 aa, synthetic construct
QQWYSSPVT

SEQ ID NO: 111 - protein, 8 aa, synthetic construct
GFNINWAN

SEQ ID NO: 112 - protein, 8 aa, synthetic construct
GFNINWAN

SEQ ID NO: 113 - protein, 8 aa, synthetic construct
GFNIYLHD

SEQ ID NO: 114 - protein, 8 aa, synthetic construct
GFNIYWSH

SEQ ID NO: 115 - protein, 8 aa, synthetic construct
ISPPYDYT

SEQ ID NO: 116 - protein, 8 aa, synthetic construct
IIPAIDYT

SEQ ID NO: 117 - protein, 8 aa, synthetic construct
ISSFEGYT

SEQ ID NO: 118 - protein, 10 aa, synthetic construct
SRSYSYYFDY

SEQ ID NO: 119 - protein, 10 aa, synthetic construct
SRRDGYYFDY

SEQ ID NO: 120 - protein, 10 aa, synthetic construct
SRSYSYYMDY

SEQ ID NO: 121 - protein, 11 aa, synthetic construct
QQSYGSGSPWT

SEQ ID NO: 122 - protein, 9 aa, synthetic construct
QQTYYSPWT

SEQ ID NO: 123 - protein, 9 aa, synthetic construct
QQYYYPPIT

SEQ ID NO: 124 - protein, 8 aa, synthetic construct
GFNIVGGG

SEQ ID NO: 125 - protein, 8 aa, synthetic construct
GFNIRSYA

SEQ ID NO: 126 - protein, 8 aa, synthetic construct
GFNVSHTG

SEQ ID NO: 127 - protein, 8 aa, synthetic construct
IYPQGDYT

SEQ ID NO: 128 - protein, 8 aa, synthetic construct
VGPGKGYT

SEQ ID NO: 129 - protein, 11 aa, synthetic construct
SRDSSYLAFDY

SEQ ID NO: 130 - protein, 13 aa, synthetic construct
SRNFQSTSHAFDY

SEQ ID NO: 131 - protein, 10 aa, synthetic construct
SRKTYYAFDY

SEQ ID NO: 132 - protein, 11 aa, synthetic construct
QQSYYYFRPIT

SEQ ID NO: 133 - protein, 10 aa, synthetic construct
QQASYYYPLT

SEQ ID NO: 134 - protein, 10 aa, synthetic construct
QQKSEYSPWT

SEQ ID NO: 135 - protein, 9 aa, synthetic construct
QQSGYIPFT

SEQ ID NO: 136 - protein, 10 aa, synthetic construct
QQGAYYRPFT

SEQ ID NO: 137 - protein, 8 aa, synthetic construct
GFNLSYSD

SEQ ID NO: 138 - protein, 8 aa, synthetic construct
GFNISASG

SEQ ID NO: 139 - protein, 8 aa, synthetic construct
GFNIYRYG

SEQ ID NO: 140 - protein, 8 aa, synthetic construct
GFNIYGTM

SEQ ID NO: 141 - protein, 8 aa, synthetic construct
GFNISYSY

SEQ ID NO: 142 - protein, 8 aa, synthetic construct
VMPDSGHT

SEQ ID NO: 143 - protein, 8 aa, synthetic construct
IHPLKPYT

SEQ ID NO: 144 - protein, 8 aa, synthetic construct
LYPYGYST

SEQ ID NO: 145 - protein, 8 aa, synthetic construct
FKPDSYNT

SEQ ID NO: 146 - protein, 8 aa, synthetic construct
LLPYDGNT

SEQ ID NO: 147 - protein, 13 aa, synthetic construct
SRATNIPVYAFDY

SEQ ID NO: 148 - protein, 13 aa, synthetic construct
SRYSSMYYYYFDY

SEQ ID NO: 149 - protein, 11 aa, synthetic construct
SRSYAYGYFAY

SEQ ID NO: 150 - protein, 13 aa, synthetic construct
SRGEVYHYYAFDY

SEQ ID NO: 151 - protein, 10 aa, synthetic construct
SRAAYSSMDV

SEQ ID NO: 152 - protein, 9 aa, synthetic construct
QQYMYSPVT

SEQ ID NO: 153 - protein, 9 aa, synthetic construct
QQSSSSPIT

SEQ ID NO: 154 - protein, 9 aa, synthetic construct
QQSSASPLT

SEQ ID NO: 155 - protein, 9 aa, synthetic construct
QQYAYSPLT

SEQ ID NO: 156 - protein, 8 aa, synthetic construct
GFNVSAYW

SEQ ID NO: 157 - protein, 8 aa, synthetic construct
GFNISGYG

SEQ ID NO: 158 - protein, 8 aa, synthetic construct
GFNVSSVG

SEQ ID NO: 159 - protein, 8 aa, synthetic construct
GFNVSSYG

SEQ ID NO: 160 - protein, 8 aa, synthetic construct
IYGGSGYT

SEQ ID NO: 161 - protein, 8 aa, synthetic construct
LYGGSDYT

SEQ ID NO: 162 - protein, 8 aa, synthetic construct
IYGTSDYT

SEQ ID NO: 163 - protein, 8 aa, synthetic construct
IAPRRDYT

SEQ ID NO: 164 - protein, 12 aa, synthetic construct
SRTHSYWSAFDY

SEQ ID NO: 165 - protein, 10 aa, synthetic construct
SRTVRYAFDY

SEQ ID NO: 166 - protein, 10 aa, synthetic construct
SRSSRYSMDY

SEQ ID NO: 167 - protein, 10 aa, synthetic construct
SRKSSYYFDY

SEQ ID NO: 168 - protein, 9 aa, synthetic construct
QQYSYYPIT

SEQ ID NO: 169 - protein, 9 aa, synthetic construct
QQYSYTPVT

SEQ ID NO: 170 - protein, 9 aa, synthetic construct
QQYSYEPVT

SEQ ID NO: 171 - protein, 10 aa, synthetic construct
QQYAYYSPVT

SEQ ID NO: 172 - protein, 9 aa, synthetic construct
QQYEYYPMT

SEQ ID NO: 173 - protein, 8 aa, synthetic construct
GFNFSYGY

SEQ ID NO: 174 - protein, 8 aa, synthetic construct
GFNVWGPG

SEQ ID NO: 175 - protein, 8 aa, synthetic construct
GFNVSGSQ

SEQ ID NO: 176 - protein, 8 aa, synthetic construct
GFNIYGQM

SEQ ID NO: 177 - protein, 8 aa, synthetic construct
GFNVMYST

SEQ ID NO: 178 - protein, 8 aa, synthetic construct
ISGYTGNT

SEQ ID NO: 179 - protein, 8 aa, synthetic construct
IHPFSGNT

SEQ ID NO: 180 - protein, 8 aa, synthetic construct
IPGWSGYT

SEQ ID NO: 181 - protein, 8 aa, synthetic construct
LSPFSGNT

SEQ ID NO: 182 - protein, 8 aa, synthetic construct
IYSWSDYT

SEQ ID NO: 183 - protein, 16 aa, synthetic construct
SRAASLSSSYYSAFDV

SEQ ID NO: 184 - protein, 11 aa, synthetic construct
SRGYSYSAMDY

SEQ ID NO: 185 - protein, 11 aa, synthetic construct
SRGYSYFAMDY

SEQ ID NO: 186 - protein, 14 aa, synthetic construct
SRNISYEQSSAFDY

SEQ ID NO: 187 - protein, 11 aa, synthetic construct
SRGYAHNSFDY

SEQ ID NO: 188 - protein, 9 aa, synthetic construct
QQYSFYPFT

SEQ ID NO: 189 - protein, 11 aa, synthetic construct
QQYSAYYQPIT

SEQ ID NO: 190 - protein, 9 aa, synthetic construct
QQYEYVPHT

SEQ ID NO: 191 - protein, 9 aa, synthetic construct
QQYSYMPIT

SEQ ID NO: 192 - protein, 9 aa, synthetic construct
QQYAYYPVT

SEQ ID NO: 193 - protein, 9 aa, synthetic construct
QQYDYRPVT

SEQ ID NO: 194 - protein, 9 aa, synthetic construct
QQYDFTPMT

SEQ ID NO: 195 - protein, 10 aa, synthetic construct
QQYSSSSPVT

SEQ ID NO: 196 - protein, 7 aa, synthetic construct
GFNFGSY

SEQ ID NO: 197 - protein, 8 aa, synthetic construct
GFNISDSY

SEQ ID NO: 198 - protein, 8 aa, synthetic construct
GFNIFSDQ

SEQ ID NO: 199 - protein, 8 aa, synthetic construct
GFNLSYSY

SEQ ID NO: 200 - protein, 8 aa, synthetic construct
GFNISYGY

SEQ ID NO: 201 - protein, 8 aa, synthetic construct
GFNISYQH

SEQ ID NO: 202 - protein, 8 aa, synthetic construct
GFNLSGYY

SEQ ID NO: 203 - protein, 8 aa, synthetic construct
GFNVSGQY

SEQ ID NO: 204 - protein, 8 aa, synthetic construct
GFNVSTSG

SEQ ID NO: 205 - protein, 8 aa, synthetic construct
GFNISYAK

SEQ ID NO: 206 - protein, 8 aa, synthetic construct
GFNFSSYV

SEQ ID NO: 207 - protein, 8 aa, synthetic construct
ISGYSGNT

SEQ ID NO: 208 - protein, 8 aa, synthetic construct
FSPYSSNT

SEQ ID NO: 209 - protein, 9 aa, synthetic construct
FMPYDSYYT

SEQ ID NO: 210 - protein, 8 aa, synthetic construct
ISGFSGNT

SEQ ID NO: 211 - protein, 8 aa, synthetic construct
FHYGSGNT

SEQ ID NO: 212 - protein, 8 aa, synthetic construct
FMPYQGST

SEQ ID NO: 213 - protein, 8 aa, synthetic construct
FSPYSGYT

SEQ ID NO: 214 - protein, 8 aa, synthetic construct
ISPVSGNT

SEQ ID NO: 215 - protein, 8 aa, synthetic construct
IYGAYSGT

SEQ ID NO: 216 - protein, 8 aa, synthetic construct
LTYWGGYT

SEQ ID NO: 217 - protein, 8 aa, synthetic construct
VYPDSGGT

SEQ ID NO: 218 - protein, 13 aa, synthetic construct
SRSNQSAYSYMDY

SEQ ID NO: 219 - protein, 13 aa, synthetic construct
SRSQFTFYQYFDY

SEQ ID NO: 220 - protein, 11 aa, synthetic construct
SRMSVRNAFDY

SEQ ID NO: 221 - protein, 12 aa, synthetic construct
SRSDSYYTAMDY

SEQ ID NO: 222 - protein, 10 aa, synthetic construct
SRSNYYYLDY

SEQ ID NO: 223 - protein, 14 aa, synthetic construct
SRANIYSSHSFFDY

SEQ ID NO: 224 - protein, 13 aa, synthetic construct
SRTHSSIYHSFDY

SEQ ID NO: 225 - protein, 14 aa, synthetic construct
SRPMKTSYYGAFDY

SEQ ID NO: 226 - protein, 14 aa, synthetic construct
SRSQSYTYWSAMDY

SEQ ID NO: 227 - protein, 11 aa, synthetic construct
SRGEYGTYMDY

SEQ ID NO: 228 - protein, 11 aa, synthetic construct
SRTSSYYAFDY

SEQ ID NO: 229 - protein, 8 aa, synthetic construct
QQSSYTPI

SEQ ID NO: 230 - protein, 9 aa, synthetic construct
QQYAYYPIT

SEQ ID NO: 231 - protein, 9 aa, synthetic construct
QQYEYYPIT

SEQ ID NO: 232 - protein, 9 aa, synthetic construct
QQYTYYPIT

SEQ ID NO: 233 - protein, 9 aa, synthetic construct
QQSSVEPWT

SEQ ID NO: 234 - protein, 8 aa, synthetic construct
GFNISQGG

SEQ ID NO: 235 - protein, 8 aa, synthetic construct
GFNISSTG

SEQ ID NO: 236 - protein, 8 aa, synthetic construct
GFNFFSTV

SEQ ID NO: 237 - protein, 8 aa, synthetic construct
GFNLHGYL

SEQ ID NO: 238 - protein, 8 aa, synthetic construct
GFNLSTHV

SEQ ID NO: 239 - protein, 8 aa, synthetic construct
GFNVSYYS

SEQ ID NO: 240 - protein, 8 aa, synthetic construct
VYPGGGQT

SEQ ID NO: 241 - protein, 8 aa, synthetic construct
LLGGSGNT

SEQ ID NO: 242 - protein, 8 aa, synthetic construct
IYPWSGST

SEQ ID NO: 243 - protein, 8 aa, synthetic construct
IYPPNGYT

SEQ ID NO: 244 - protein, 8 aa, synthetic construct
FYPYVGYT

SEQ ID NO: 245 - protein, 8 aa, synthetic construct
IYPWNDYT

SEQ ID NO: 246 - protein, 11 aa, synthetic construct
SRGYDYSAFDY

SEQ ID NO: 247 - protein, 11 aa, synthetic construct
SRGLQYSAMDY

SEQ ID NO: 248 - protein, 12 aa, synthetic construct
SRSRSSNYYFDV

SEQ ID NO: 249 - protein, 11 aa, synthetic construct
SRGVDYAYLDY

SEQ ID NO: 250 - protein, 11 aa, synthetic construct
SRGYRYQYMDV

SEQ ID NO: 251 - protein, 10 aa, synthetic construct
SRGSYYSFDY

SEQ ID NO: 252 - protein, 9 aa, synthetic construct
QQIYTSPIT

SEQ ID NO: 253 - protein, 9 aa, synthetic construct
QQRAYFPIT

SEQ ID NO: 254 - protein, 10 aa, synthetic construct
QQQYAYTPIT

SEQ ID NO: 255 - protein, 9 aa, synthetic construct
QQIHYKPLT

SEQ ID NO: 256 - protein, 8 aa, synthetic construct
GFNINNTY

SEQ ID NO: 257 - protein, 8 aa, synthetic construct
GFNFITTG

SEQ ID NO: 258 - protein, 8 aa, synthetic construct
GFNFSDYG

SEQ ID NO: 259 - protein, 8 aa, synthetic construct
GFNVWSYG

SEQ ID NO: 260 - protein, 8 aa, synthetic construct
GFNVAWYS

SEQ ID NO: 261 - protein, 8 aa, synthetic construct
IGPGSDYT

SEQ ID NO: 262 - protein, 8 aa, synthetic construct
LIPASGYT

SEQ ID NO: 263 - protein, 8 aa, synthetic construct
VTPDGSYT

SEQ ID NO: 264 - protein, 8 aa, synthetic construct
VYGGSSYT

SEQ ID NO: 265 - protein, 13 aa, synthetic construct
SRTYYSYYSAMDV

SEQ ID NO: 266 - protein, 11 aa, synthetic construct
SRYYYASALDY

SEQ ID NO: 267 - protein, 10 aa, synthetic construct
SRGWSYYMDY

SEQ ID NO: 268 - protein, 10 aa, synthetic construct
SRSYGWAMDY

SEQ ID NO: 269 - protein, 11 aa, synthetic construct
SRDFYSSGMDY

SEQ ID NO: 270 - protein, 9 aa, synthetic construct
QQEWRLPIT

SEQ ID NO: 271 - protein, 9 aa, synthetic construct
QQGTSTPFT

SEQ ID NO: 272 - protein, 9 aa, synthetic construct
QQSWRYPMT

SEQ ID NO: 273 - protein, 9 aa, synthetic construct
QQSYSYPVT

SEQ ID NO: 274 - protein, 10 aa, synthetic construct
QQGWLYSPFT

SEQ ID NO: 275 - protein, 8 aa, synthetic construct
GFNVYGNQ

SEQ ID NO: 276 - protein, 8 aa, synthetic construct
GFNISRYG

SEQ ID NO: 277 - protein, 8 aa, synthetic construct
GFNIYSSW

SEQ ID NO: 278 - protein, 8 aa, synthetic construct
IYPYSGST

SEQ ID NO: 279 - protein, 8 aa, synthetic construct
IYPDSGYT

SEQ ID NO: 280 - protein, 8 aa, synthetic construct
FYPSSSYT

SEQ ID NO: 281 - protein, 8 aa, synthetic construct
FQPYSGYT

SEQ ID NO: 282 - protein, 8 aa, synthetic construct
VYGGSGYT

SEQ ID NO: 283 - protein, 13 aa, synthetic construct
SRSAYVAYSYFDY

SEQ ID NO: 284 - protein, 11 aa, synthetic construct
SRAYLYYYLAY

SEQ ID NO: 285 - protein, 10 aa, synthetic construct
SRKYYEAMDY

SEQ ID NO: 286 - protein, 10 aa, synthetic construct
SREYTYYFDY

SEQ ID NO: 287 - protein, 11 aa, synthetic construct
SRAHSSYYVDY

SEQ ID NO: 288 - protein, 10 aa, synthetic construct
QQGYFYYPNT

SEQ ID NO: 289 - protein, 8 aa, synthetic construct
GFNIGYYG

SEQ ID NO: 290 - protein, 8 aa, synthetic construct
VYPGGGYT

SEQ ID NO: 291 - protein, 10 aa, synthetic construct
SRYYYYGFDY

SEQ ID NO: 292 - protein, 9 aa, synthetic construct
QQHYYSPVT

SEQ ID NO: 293 - protein, 9 aa, synthetic construct
QQHYYSPVT

SEQ ID NO: 294 - protein, 8 aa, synthetic construct
IYPDYDYT

SEQ ID NO: 295 - protein, 10 aa, synthetic construct
SRTYSVYMDY

SEQ ID NO: 296 - protein, 9 aa, synthetic construct
QQYAYAPFT

SEQ ID NO: 297 - protein, 8 aa, synthetic construct
GFNVSYSM

SEQ ID NO: 298 - protein, 8 aa, synthetic construct
VWGDGGVT

SEQ ID NO: 299 - protein, 10 aa, synthetic construct
SRGSYYAFDY

SEQ ID NO: 300 - protein, 9 aa, synthetic construct
QQAHMIPIT

SEQ ID NO: 301 - protein, 9 aa, synthetic construct
QQSVYDPIT

SEQ ID NO: 302 - protein, 9 aa, synthetic construct
QQSYTSPLT

SEQ ID NO: 303 - protein, 9 aa, synthetic construct
QQGQYSPFT

SEQ ID NO: 304 - skipped

SEQ ID NO: 305 - protein, 8 aa, synthetic construct
GFNFSFPG

SEQ ID NO: 306 - protein, 8 aa, synthetic construct
GFNISGSW

SEQ ID NO: 307 - protein, 8 aa, synthetic construct
GFNIYYGV

SEQ ID NO: 308 - protein, 8 aa, synthetic construct
GFNVSYEY

SEQ ID NO: 309 - skipped

SEQ ID NO: 310 - protein, 8 aa, synthetic construct
FVGYDGYT

SEQ ID NO: 311 - protein, 8 aa, synthetic construct
LYPDSDYT

SEQ ID NO: 312 - protein, 8 aa, synthetic construct
IYPDSSWT

SEQ ID NO: 313 - protein, 8 aa, synthetic construct
IYGGSDNT

SEQ ID NO: 314-315 - skipped (2 entries)

SEQ ID NO: 316 - protein, 11 aa, synthetic construct
SRDYYSFSMDY

SEQ ID NO: 317 - protein, 10 aa, synthetic construct
SRAHTYAFDY

SEQ ID NO: 318 - protein, 19 aa, synthetic construct
SRDQDFHYMNYYLSYALDY

SEQ ID NO: 319 - protein, 10 aa, synthetic construct
SRPLGSYFDY

SEQ ID NO: 320 - protein, 9 aa, synthetic construct
QQYWYLPTT

SEQ ID NO: 321 - protein, 8 aa, synthetic construct
GFNISWYD

SEQ ID NO: 322 - protein, 8 aa, synthetic construct
IEPSVGYT

SEQ ID NO: 323 - protein, 11 aa, synthetic construct
SRSYPYYYFDY

SEQ ID NO: 324 - protein, 240 aa, synthetic construct
DIQMTQSPSSLSASVGDRVTITCRASQDVNTAVAWYQQKPGKAPKLLIYSASFLYSGVPSRFSGSRSGTDFTLTISSLQPEDFATYYCQQYDYAPITFGQGTKVEIKRTGGGSGGGGSGGGASEVQLVESGGGLVQPGGSLRLSCAASGFNISWYQMHWVRQAPGKGLEWVALVTPYSGYTYYADSVKGRFTISADTSKNTAYLQMNSLRAEDTAVYYCSRSYTDGFDYWGQGTLVTVSS

SEQ ID NO: 325 - protein, 246 aa, synthetic construct
DIQMTQSPSSLSASVGDRVTITCRASQDVNTAVAWYQQKPGKAPKLLIYSASFLYSGVPSRFSGSRSGTDFTLTISSLQPEDFATYYCQQSPYYYLPITFGQGTKVEIKRTGGGSGGGGSGGGASEVQLVESGGGLVQPGGSLRLSCAASGFNVSWSYMHWVRQAPGKGLEWVANIYGDSGYTHYADSVKGRFTISADTSKNTAYLQMNSLRAEDTAVYYCSRGQWEASYYAMDYWGQGTLVTVSS

SEQ ID NO: 326 - protein, 240 aa, synthetic construct
DIQMTQSPSSLSASVGDRVTITCRASQDVNTAVAWYQQKPGKAPKLLIYSASFLYSGVPSRFSGSRSGTDFTLTISSLQPEDFATYYCQQYYYSPVTFGQGTKVEIKRTGGGSGGGGSGGGASEVQLVESGGGLVQPGGSLRLSCAASGFNISWNQMHWVRQAPGKGLEWVALVSPYSGYTYYADSVKGRFTISADTSKNTAYLQMNSLRAEDTAVYYCSRSDYYAMDYWGQGTLVTVSS

SEQ ID NO: 327 - protein, 241 aa, synthetic construct
DIQMTQSPSSLSASVGDRVTITCRASQDVNTAVAWYQQKPGKAPKLLIYSASFLYSGVPSRFSGSRSGTDFTLTISSLQPEDFATYYCQQHYGNPFTFGQGTKVEIKRTGGGSGGGGSGGGASEVQLVESGGGLVQPGGSLRLSCAASGFNVGYYGMHWVRQAPGKGLEWVAFVSGMEGYTSYADSVKGRFTISADTSKNTAYLQMNSLRAEDTAVYYCSRDIYGYAMDVWGQGTLVTVSS

SEQ ID NO: 328 - protein, 243 aa, synthetic construct
DIQMTQSPSSLSASVGDRVTITCRASQDVNTAVAWYQQKPGKAPKLLIYSASFLYSGVPSRFSGSRSGTDFTLTISSLQPEDFATYYCQQSYYSPPTFGQGTKVEIKRTGGGSGGGGSGGGASEVQLVESGGGLVQPGGSLRLSCAASGFNITSSYIHWVRQAPGKGLEWVAYISPADGYNRYADSVKGRFTISADTSKNTAYLQMNSLRAEDTAVYYCSRTDSTAYTAMDVWGQGTLVTVSS

SEQ ID NO: 329 - protein, 243 aa, synthetic construct
DIQMTQSPSSLSASVGDRVTITCRASQDVNTAVAWYQQKPGKAPKLLIYSASFLYSGVPSRFSGSRSGTDFTLTISSLQPEDFATYYCQQYYSYPPTFGQGTKVEIKRTGGGSGGGGSGGGASEVQLVESGGGLVQPGGSLRLSCAASGFNINSSYIHWVRQAPGKGLEWVAYISPTDGYYRYADSVKGRFTISADTSKNTAYLQMNSLRAEDTAVYYCSRTSDTSYAAMDVWGQGTLVTVSS

SEQ ID NO: 330 - protein, 243 aa, synthetic construct
DIQMTQSPSSLSASVGDRVTITCRASQDVNTAVAWYQQKPGKAPKLLIYSASFLYSGVPSRFSGSRSGTDFTLTISSLQPEDFATYYCQQYYYYPPTFGQGTKVEIKRTGGGSGGGGSGGGASEVQLVESGGGLVQPGGSLRLSCAASGFNISTSYIHWVRQAPGKGLEWVATIDPNDGYSRYADSVKGRFTISADTSKNTAYLQMNSLRAEDTAVYYCSRTNNTAADAMDVWGQGTLVTVSS

SEQ ID NO: 331 - protein, 242 aa, synthetic construct
DIQMTQSPSSLSASVGDRVTITCRASQDVNTAVAWYQQKPGKAPKLLIYSASFLYSGVPSRFSGSRSGTDFTLTISSLQPEDFATYYCQQSGYAPITFGQGTKVEIKRTGGGSGGGGSGGGASEVQLVESGGGLVQPGGSLRLSCAASGFNISYYSMHWVRQAPGKGLEWVADVDPDSDYTEYADSVKGRFTISADTSKNTAYLQMNSLRAEDTAVYYCSRSWIHMFSMDYWGQGTLVTVSS

SEQ ID NO: 332 - protein, 241 aa, synthetic construct
DIQMTQSPSSLSASVGDRVTITCRASQDVNTAVAWYQQKPGKAPKLLIYSASFLYSGVPSRFSGSRSGTDFTLTISSLQPEDFATYYCQQYSYAPITFGQGTKVEIKRTGGGSGGGGSGGGASEVQLVESGGGLVQPGGSLRLSCAASGFNIGYYTMHWVRQAPGKGLEWVAEVSPWSYSTSYADSVKGRFTISADTSKNTAYLQMNSLRAEDTAVYYCSRDHWDEAFDVWGQGTLVTVSS

SEQ ID NO: 333 - protein, 243 aa, synthetic construct
DIQMTQSPSSLSASVGDRVTITCRASQDVNTAVAWYQQKPGKAPKLLIYSASFLYSGVPSRFSGSRSGTDFTLTISSLQPEDFATYYCQQSLYGPFTFGQGTKVEIKRTGGGSGGGGSGGGASEVQLVESGGGLVQPGGSLRLSCAASGFNIAYEYMHWVRQAPGKGLEWVALIGPDSGYTYYADSVKGRFTISADTSKNTAYLQMNSLRAEDTAVYYCSRVWYYSTYGMDYWGQGTLVTVSS

SEQ ID NO: 334 - protein, 241 aa, synthetic construct
DIQMTQSPSSLSASVGDRVTITCRASQDVNTAVAWYQQKPGKAPKLLIYSASFLYSGVPSRFSGSRSGTDFTLTISSLQPEDFATYYCQQYSYSPITFGQGTKVEIKRTGGGSGGGGSGGGASEVQLVESGGGLVQPGGSLRLSCAASGFNLFGYGMHWVRQAPGKGLEWVAEIGPYYYYTSYADSVKGRFTISADTSKNTAYLQMNSLRAEDTAVYYCSRENYDMAMDYWGQGTLVTVSS

SEQ ID NO: 335 - protein, 241 aa, synthetic construct
DIQMTQSPSSLSASVGDRVTITCRASQDVNTAVAWYQQKPGKAPKLLIYSASFLYSGVPSRFSGSRSGTDFTLTISSLQPEDFATYYCQQSGYQPDTFGQGTKVEIKRTGGGSGGGGSGGGASEVQLVESGGGLVQPGGSLRLSCAASGFNISWYAMHWVRQAPGKGLEWVAEIWPDSDWTYYADSVKGRFTISADTSKNTAYLQMNSLRAEDTAVYYCSRYYYSSAFDVWGQGTLVTVSS

SEQ ID NO: 336 - protein, 240 aa, synthetic construct
DIQMTQSPSSLSASVGDRVTITCRASQDVNTAVAWYQQKPGKAPKLLIYSASFLYSGVPSRFSGSRSGTDFTLTISSLQPEDFATYYCQQYLYQPWTFGQGTKVEIKRTGGGSGGGGSGGGASEVQLVESGGGLVQPGGSLRLSCAASGFNIDYYGMHWVRQAPGKGLEWVASLYGGSDSTDYADSVKGRFTISADTSKNTAYLQMNSLRAEDTAVYYCSRQYSAYFDYWGQGTLVTVSS

SEQ ID NO: 337 - protein, 241 aa, synthetic construct
DIQMTQSPSSLSASVGDRVTITCRASQDVNTAVAWYQQKPGKAPKLLIYSASFLYSGVPSRFSGSRSGTDFTLTISSLQPEDFATYYCQQGLYYPWTFGQGTKVEIKRTGGGSGGGGSGGGASEVQLVESGGGLVQPGGSLRLSCAASGFNVSYSSIHWVRQAPGKGLEWVAEIWPDSGQTWYADSVKGRFTISADTSKNTAYLQMNSLRAEDTAVYYCSRSSYFDAMDYWGQGTLVTVSS

SEQ ID NO: 338 - protein, 240 aa, synthetic construct
DIQMTQSPSSLSASVGDRVTITCRASQDVNTAVAWYQQKPGKAPKLLIYSASFLYSGVPSRFSGSRSGTDFTLTISSLQPEDFATYYCQQWYSSPVTFGQGTKVEIKRTGGGSGGGGSGGGASEVQLVESGGGLVQPGGSLRLSCAASGFNINWANMHWVRQAPGKGLEWVAQISPPYDYTNYADSVKGRFTISADTSKNTAYLQMNSLRAEDTAVYYCSRSYSYYFDYWGQGTLVTVSS

SEQ ID NO: 339 - protein, 240 aa, synthetic construct
DIQMTQSPSSLSASVGDRVTITCRASQDVNTAVAWYQQKPGKAPKLLIYSASFLYSGVPSRFSGSRSGTDFTLTISSLQPEDFATYYCQQYYSRPVTFGQGTKVEIKRTGGGSGGGGSGGGASEVQLVESGGGLVQPGGSLRLSCAASGFNIYLHDMHWVRQAPGKGLEWVAQIIPAIDYTNYADSVKGRFTISADTSKNTAYLQMNSLRAEDTAVYYCSRRDGYYFDYWGQGTLVTVSS

SEQ ID NO: 340 - protein, 240 aa, synthetic construct
DIQMTQSPSSLSASVGDRVTITCRASQDVNTAVAWYQQKPGKAPKLLIYSASFLYSGVPSRFSGSRSGTDFTLTISSLQPEDFATYYCQQWYSSPVTFGQGTKVEIKRTGGGSGGGGSGGGASEVQLVESGGGLVQPGGSLRLSCAASGFNIYWSHMHWVRQAPGKGLEWVAIISSFEGYTYYADSVKGRFTISADTSKNTAYLQMNSLRAEDTAVYYCSRSYSYYMDYWGQGTLVTVSS

SEQ ID NO: 341 - protein, 243 aa, synthetic construct
DIQMTQSPSSLSASVGDRVTITCRASQDVNTAVAWYQQKPGKAPKLLIYSASFLYSGVPSRFSGSRSGTDFTLTISSLQPEDFATYYCQQSYGSGSPWTFGQGTKVEIKRTGGGSGGGGSGGGASEVQLVESGGGLVQPGGSLRLSCAASGFNIVGGGIHWVRQAPGKGLEWVAKIYPQGDYTYYADSVKGRFTISADTSKNTAYLQMNSLRAEDTAVYYCSRDSSYLAFDYWGQGTLVTVSS

SEQ ID NO: 342 - protein, 243 aa, synthetic construct
DIQMTQSPSSLSASVGDRVTITCRASQDVNTAVAWYQQKPGKAPKLLIYSASFLYSGVPSRFSGSRSGTDFTLTISSLQPEDFATYYCQQTYYSPWTFGQGTKVEIKRTGGGSGGGGSGGGASEVQLVESGGGLVQPGGSLRLSCAASGFNIRSYAMHWVRQAPGKGLEWVAQVGPGKGYTYYADSVKGRFTISADTSKNTAYLQMNSLRAEDTAVYYCSRNFQSTSHAFDYWGQGTLVTVSS

SEQ ID NO: 343 - protein, 240 aa, synthetic construct
DIQMTQSPSSLSASVGDRVTITCRASQDVNTAVAWYQQKPGKAPKLLIYSASFLYSGVPSRFSGSRSGTDFTLTISSLQPEDFATYYCQQYYYPPITFGQGTKVEIKRTGGGSGGGGSGGGASEVQLVESGGGLVQPGGSLRLSCAASGFNVSHTGMHWVRQAPGKGLEWVAVVGPGKGYTYYADSVKGRFTISADTSKNTAYLQMNSLRAEDTAVYYCSRKTYYAFDYWGQGTLVTVSS

SEQ ID NO: 344 - protein, 245 aa, synthetic construct
DIQMTQSPSSLSASVGDRVTITCRASQDVNTAVAWYQQKPGKAPKLLIYSASFLYSGVPSRFSGSRSGTDFTLTISSLQPEDFATYYCQQSYYYFRPITFGQGTKVEIKRTGGGSGGGGSGGGASEVQLVESGGGLVQPGGSLRLSCAASGFNLSYSDIHWVRQAPGKGLEWVAVVMPDSGHTNYADSVKGRFTISADTSKNTAYLQMNSLRAEDTAVYYCSRATNIPVYAFDYWGQGTLVTVSS

SEQ ID NO: 345 - protein, 244 aa, synthetic construct
DIQMTQSPSSLSASVGDRVTITCRASQDVNTAVAWYQQKPGKAPKLLIYSASFLYSGVPSRFSGSRSGTDFTLTISSLQPEDFATYYCQQASYYYPLTFGQGTKVEIKRTGGGSGGGGSGGGASEVQLVESGGGLVQPGGSLRLSCAASGFNISASGMHWVRQAPGKGLEWVADIHPLKPYTNYADSVKGRFTISADTSKNTAYLQMNSLRAEDTAVYYCSRYSSMYYYYFDYWGQGTLVTVSS

SEQ ID NO: 346 - protein, 242 aa, synthetic construct
DIQMTQSPSSLSASVGDRVTITCRASQDVNTAVAWYQQKPGKAPKLLIYSASFLYSGVPSRFSGSRSGTDFTLTISSLQPEDFATYYCQQKSEYSPWTFGQGTKVEIKRTGGGSGGGGSGGGASEVQLVESGGGLVQPGGSLRLSCAASGFNIYRYGIHWVRQAPGKGLEWVAVLYPYGYSTSYADSVKGRFTISADTSKNTAYLQMNSLRAEDTAVYYCSRSYAYGYFAYWGQGTLVTVSS

SEQ ID NO: 347 - protein, 243 aa, synthetic construct
DIQMTQSPSSLSASVGDRVTITCRASQDVNTAVAWYQQKPGKAPKLLIYSASFLYSGVPSRFSGSRSGTDFTLTISSLQPEDFATYYCQQSGYIPFTFGQGTKVEIKRTGGGSGGGGSGGGASEVQLVESGGGLVQPGGSLRLSCAASGFNIYGTMMHWVRQAPGKGLEWVAQFKPDSYNTYYADSVKGRFTISADTSKNTAYLQMNSLRAEDTAVYYCSRGEVYHYYAFDYWGQGTLVTVSS

SEQ ID NO: 348 - protein, 241 aa, synthetic construct
DIQMTQSPSSLSASVGDRVTITCRASQDVNTAVAWYQQKPGKAPKLLIYSASFLYSGVPSRFSGSRSGTDFTLTISSLQPEDFATYYCQQGAYYRPFTFGQGTKVEIKRTGGGSGGGGSGGGASEVQLVESGGGLVQPGGSLRLSCAASGFNISYSYMHWVRQAPGKGLEWVATLLPYDGNTYYADSVKGRFTISADTSKNTAYLQMNSLRAEDTAVYYCSRAAYSSMDVWGQGTLVTVSS

SEQ ID NO: 349 - protein, 242 aa, synthetic construct
DIQMTQSPSSLSASVGDRVTITCRASQDVNTAVAWYQQKPGKAPKLLIYSASFLYSGVPSRFSGSRSGTDFTLTISSLQPEDFATYYCQQYMYSPVTFGQGTKVEIKRTGGGSGGGGSGGGASEVQLVESGGGLVQPGGSLRLSCAASGFNVSAYWMHWVRQAPGKGLEWVAQIYGGSGYTMYADSVKGRFTISADTSKNTAYLQMNSLRAEDTAVYYCSRTHSYWSAFDYWGQGTLVTVSS

SEQ ID NO: 350 - protein, 240 aa, synthetic construct
DIQMTQSPSSLSASVGDRVTITCRASQDVNTAVAWYQQKPGKAPKLLIYSASFLYSGVPSRFSGSRSGTDFTLTISSLQPEDFATYYCQQSSSSPITFGQGTKVEIKRTGGGSGGGGSGGGASEVQLVESGGGLVQPGGSLRLSCAASGFNISGYGMHWVRQAPGKGLEWVAYLYGGSDYTNYADSVKGRFTISADTSKNTAYLQMNSLRAEDTAVYYCSRTVRYAFDYWGQGTLVTVSS

SEQ ID NO: 351 - protein, 240 aa, synthetic construct
DIQMTQSPSSLSASVGDRVTITCRASQDVNTAVAWYQQKPGKAPKLLIYSASFLYSGVPSRFSGSRSGTDFTLTISSLQPEDFATYYCQQSSASPLTFGQGTKVEIKRTGGGSGGGGSGGGASEVQLVESGGGLVQPGGSLRLSCAASGFNVSSVGMHWVRQAPGKGLEWVAYIYGTSDYTYYADSVKGRFTISADTSKNTAYLQMNSLRAEDTAVYYCSRSSRYSMDYWGQGTLVTVSS

SEQ ID NO: 352 - protein, 240 aa, synthetic construct
DIQMTQSPSSLSASVGDRVTITCRASQDVNTAVAWYQQKPGKAPKLLIYSASFLYSGVPSRFSGSRSGTDFTLTISSLQPEDFATYYCQQYAYSPLTFGQGTKVEIKRTGGGSGGGGSGGGASEVQLVESGGGLVQPGGSLRLSCAASGFNVSSYGMHWVRQAPGKGLEWVAFIAPRRDYTSYADSVKGRFTISADTSKNTAYLQMNSLRAEDTAVYYCSRKSSYYFDYWGQGTLVTVSS

SEQ ID NO: 353 - protein, 246 aa, synthetic construct
DIQMTQSPSSLSASVGDRVTITCRASQDVNTAVAWYQQKPGKAPKLLIYSASFLYSGVPSRFSGSRSGTDFTLTISSLQPEDFATYYCQQYSYYPITFGQGTKVEIKRTGGGSGGGGSGGGASEVQLVESGGGLVQPGGSLRLSCAASGFNFSYGYMHWVRQAPGKGLEWVAWISGYTGNTYYADSVKGRFTISADTSKNTAYLQMNSLRAEDTAVYYCSRAASLSSSYYSAFDVWGQGTLVTVSS

SEQ ID NO: 354 - protein, 241 aa, synthetic construct
DIQMTQSPSSLSASVGDRVTITCRASQDVNTAVAWYQQKPGKAPKLLIYSASFLYSGVPSRFSGSRSGTDFTLTISSLQPEDFATYYCQQYSYTPVTFGQGTKVEIKRTGGGSGGGGSGGGASEVQLVESGGGLVQPGGSLRLSCAASGFNVWGPGMHWVRQAPGKGLEWVARIHPFSGNTYYADSVKGRFTISADTSKNTAYLQMNSLRAEDTAVYYCSRGYSYSAMDYWGQGTLVTVSS

SEQ ID NO: 355 - protein, 241 aa, synthetic construct
DIQMTQSPSSLSASVGDRVTITCRASQDVNTAVAWYQQKPGKAPKLLIYSASFLYSGVPSRFSGSRSGTDFTLTISSLQPEDFATYYCQQYSYEPVTFGQGTKVEIKRTGGGSGGGGSGGGASEVQLVESGGGLVQPGGSLRLSCAASGFNVSGSQMHWVRQAPGKGLEWVARIPGWSGYTYYADSVKGRFTISADTSKNTAYLQMNSLRAEDTAVYYCSRGYSYFAMDYWGQGTLVTVSS

SEQ ID NO: 356 - protein, 245 aa, synthetic construct
DIQMTQSPSSLSASVGDRVTITCRASQDVNTAVAWYQQKPGKAPKLLIYSASFLYSGVPSRFSGSRSGTDFTLTISSLQPEDFATYYCQQYAYYSPVTFGQGTKVEIKRTGGGSGGGGSGGGASEVQLVESGGGLVQPGGSLRLSCAASGFNIYGQMMHWVRQAPGKGLEWVAFLSPFSGNTYYADSVKGRFTISADTSKNTAYLQMNSLRAEDTAVYYCSRNISYEQSSAFDYWGQGTLVTVSS

SEQ ID NO: 357 - protein, 241 aa, synthetic construct
DIQMTQSPSSLSASVGDRVTITCRASQDVNTAVAWYQQKPGKAPKLLIYSASFLYSGVPSRFSGSRSGTDFTLTISSLQPEDFATYYCQQYEYYPMTFGQGTKVEIKRTGGGSGGGGSGGGASEVQLVESGGGLVQPGGSLRLSCAASGFNVMYSTMHWVRQAPGKGLEWVASIYSWSDYTYYADSVKGRFTISADTSKNTAYLQMNSLRAEDTAVYYCSRGYAHNSFDYWGQGTLVTVSS

SEQ ID NO: 358 - protein, 242 aa, synthetic construct
DIQMTQSPSSLSASVGDRVTITCRASQDVNTAVAWYQQKPGKAPKLLIYSASFLYSGVPSRFSGSRSGTDFTLTISSLQPEDFATYYCQQYSFYPFTFGQGTKVEIKRTGGGSGGGGSGGGASEVQLVESGGGLVQPGGSLRLSCAASGFNFGSYIHWVRQAPGKGLEWVAIISGYSGNTYYADSVKGRFTISADTSKNTAYLQMNSLRAEDTAVYYCSRSNQSAYSYMDYWGQGTLVTVSS

SEQ ID NO: 359 - protein, 243 aa, synthetic construct
DIQMTQSPSSLSASVGDRVTITCRASQDVNTAVAWYQQKPGKAPKLLIYSASFLYSGVPSRFSGSRSGTDFTLTISSLQPEDFATYYCQQYSYSPITFGQGTKVEIKRTGGGSGGGGSGGGASEVQLVESGGGLVQPGGSLRLSCAASGFNISDSYMHWVRQAPGKGLEWVATFSPYSSNTWYADSVKGRFTISADTSKNTAYLQMNSLRAEDTAVYYCSRSQFTFYQYFDYWGQGTLVTVSS

SEQ ID NO: 360 - protein, 244 aa, synthetic construct
DIQMTQSPSSLSASVGDRVTITCRASQDVNTAVAWYQQKPGKAPKLLIYSAYFLYSGVPSRFSGSRSGTDFTLTISSLQPEDFATYYCQQYSAYYQPITFGQGTKVEIKRTGGGSGGGGSGGGASEVQLVESGGGLVQPGGSLRLSCAASGFNIFSDQMHWVRQAPGKGLEWVAGFMPYDSYYTNYADSVKGRFTISADTSKNTAYLQMNSLRAEDTAVYYCSRMSVRNAFDYWGQGTLVTVSS

SEQ ID NO: 361 - protein, 242 aa, synthetic construct
DIQMTQSPSSLSASVGDRVTITCRASQDVNTAVAWYQQKPGKAPKLLIYSASFLYSGVPSRFSGSRSGTDFTLTISSLQPEDFATYYCQQYSYYPITFGQGTKVEIKRTGGGSGGGGSGGGASEVQLVESGGGLVQPGGSLRLSCAASGFNLSYSYMHWVRQAPGKGLEWVAVISGFSGNTYYADSVKGRFTISADTSKNTAYLQMNSLRAEDTAVYYCSRSDSYYTAMDYWGQGTLVTVSS

SEQ ID NO: 362 - protein, 240 aa, synthetic construct
DIQMTQSPSSLSASVGDRVTITCRASQDVNTAVAWYQQKPGKAPKLLIYSASFLYSGVPSRFSGSRSGTDFTLTISSLQPEDFATYYCQQYEYVPHTFGQGTKVEIKRTGGGSGGGGSGGGASEVQLVESGGGLVQPGGSLRLSCAASGFNISYGYMHWVRQAPGKGLEWVAKFHYGSGNTYYADSVKGRFTISADTSKNTAYLQMNSLRAEDTAVYYCSRSNYYYLDYWGQGTLVTVSS

SEQ ID NO: 363 - protein, 244 aa, synthetic construct
DIQMTQSPSSLSASVGDRVTITCRASQDVNTAVAWYQQKPGKAPKLLIYSASFLYSGVPSRFSGSRSGTDFTLTISSLQPEDFATYYCQQYSYMPITFGQGTKVEIKRTGGGSGGGGSGGGASEVQLVESGGGLVQPGGSLRLSCAASGFNISYQHIHWVRQAPGKGLEWVAVFMPYQGSTYYADSVKGRFTISADTSKNTAYLQMNSLRAEDTAVYYCSRANIYSSHSFFDYWGQGTLVTVSS

SEQ ID NO: 364 - protein, 243 aa, synthetic construct
DIQMTQSPSSLSASVGDRVTITCRASQDVNTAVAWYQQKPGKAPKLLIYSASFLYSGVPSRFSGSRSGTDFTLTISSLQPEDFATYYCQQYAYYPVTFGQGTKVEIKRTGGGSGGGGSGGGASEVQLVESGGGLVQPGGSLRLSCAASGFNLSGYYMHWVRQAPGKGLEWVAWFSPYSGYTYYADSVKGRFTISADTSKNTAYLQMNSLRAEDTAVYYCSRTHSSIYHSFDYWGQGTLVTVSS

SEQ ID NO: 365 - protein, 244 aa, synthetic construct
DIQMTQSPSSLSASVGDRVTITCRASQDVNTAVAWYQQKPGKAPKLLIYSASFLYSGVPSRFSGSRSGTDFTLTISSLQPEDFATYYCQQYSYMPITFGQGTKVEIKRTGGGSGGGGSGGGASEVQLVESGGGLVQPGGSLRLSCAASGFNVSGQYMHWVRQAPGKGLEWVAVISPVSGNTYYADSVKGRFTISADTSKNTAYLQMNSLRAEDTAVYYCSRPMKTSYYGAFDYWGQGTLVTVSS

SEQ ID NO: 366 - protein, 244 aa, synthetic construct
DIQMTQSPSSLSASVGDRVTITCRASQDVNTAVAWYQQKPGKAPKLLIYSASFLYSGVPSRFSGSRSGTDFTLTISSLQPEDFATYYCQQYDYRPVTFGQGTKVEIKRTGGGSGGGGSGGGASEVQLVESGGGLVQPGGSLRLSCAASGFNVSTSGMHWVRQAPGKGLEWVAFIYGAYSGTYYADSVKGRFTISADTSKNTAYLQMNSLRAEDTAVYYCSRSQSYTYWSAMDYWGQGTLVTVSS

SEQ ID NO: 367 - protein, 241 aa, synthetic construct
DIQMTQSPSSLSASVGDRVTITCRASQDVNTAVAWYQQKPGKAPKLLIYSASFLYSGVPSRFSGSRSGTDFTLTISSLQPEDFATYYCQQYDFTPMTFGQGTKVEIKRTGGGSGGGGSGGGASEVQLVESGGGLVQPGGSLRLSCAASGFNISYAKMHWVRQAPGKGLEWVAYLTYWGGYTNYADSVKGRFTISADTSKNTAYLQMNSLRAEDTAVYYCSRGEYGTYMDYWGQGTLVTVSS

SEQ ID NO: 368 - protein, 242 aa, synthetic construct
DIQMTQSPSSLSASVGDRVTITCRASQDVNTAVAWYQQKPGKAPKLLIYSASFLYSGVPSRFSGSRSGTDFTLTISSLQPEDFATYYCQQYSSSSPVTFGQGTKVEIKRTGGGSGGGGSGGGASEVQLVESGGGLVQPGGSLRLSCAASGFNFSSYVMHWVRQAPGKGLEWVAVVYPDSGGTYYADSVKGRFTISADTSKNTAYLQMNSLRAEDTAVYYCSRTSSYYAFDYWGQGTLVTVSS

SEQ ID NO: 369 - protein, 241 aa, synthetic construct
DIQMTQSPSSLSASVGDRVTITCRASQDVNTAVAWYQQKPGKAPKLLIYSASFLYSGVPSRFSGSRSGTDFTLTISSLQPEDFATYYCQQSSYTPITFGQGTKVEIKRTGGGSGGGGSGGGASEVQLVESGGGLVQPGGSLRLSCAASGFNISQGGIHWVRQAPGKGLEWVAYVYPGGGQTNYADSVKGRFTISADTSKNTAYLQMNSLRAEDTAVYYCSRGYDYSAFDYWGQGTLVTVSS

SEQ ID NO: 370 - protein, 241 aa, synthetic construct
DIQMTQSPSSLSASVGDRVTITCRASQDVNTAVAWYQQKPGKAPKLLIYSASFLYSGVPSRFSGSRSGTDFTLTISSLQPEDFATYYCQQYAYYPITFGQGTKVEIKRTGGGSGGGGSGGGASEVQLVESGGGLVQPGGSLRLSCAASGFNISSTGMHWVRQAPGKGLEWVAELLGGSGNTNYADSVKGRFTISADTSKNTAYLQMNSLRAEDTAVYYCSRGLQYSAMDYWGQGTLVTVSS

SEQ ID NO: 371 - protein, 242 aa, synthetic construct
DIQMTQSPSSLSASVGDRVTITCRASQDVNTAVAWYQQKPGKAPKLLIYSASFLYSGVPSRFSGSRSGTDFTLTISSLQPEDFATYYCQQYEYYPITFGQGTKVEIKRTGGGSGGGGSGGGASEVQLVESGGGLVQPGGSLRLSCAASGFNFFSTVIHWVRQAPGKGLEWVAEIYPWSGSTYYADSVKGRFTISADTSKNTAYLQMNSLRAEDTAVYYCSRSRSSNYYFDVWGQGTLVTVSS

SEQ ID NO: 372 - protein, 241 aa, synthetic construct
DIQMTQSPSSLSASVGDRVTITCRASQDVNTAVAWYQQKPGKAPKLLIYSASFLYSGVPSRFSGSRSGTDFTLTISSLQPEDFATYYCQQYTYYPITFGQGTKVEIKRTGGGSGGGGSGGGASEVQLVESGGGLVQPGGSLRLSCAASGFNLHGYLMHWVRQAPGKGLEWVAFIYPPNGYTYYADSVKGRFTISADTSKNTAYLQMNSLRAEDTAVYYCSRGVDYAYLDYWGQGTLVTVSS

SEQ ID NO: 373 - protein, 241 aa, synthetic construct
DIQMTQSPSSLSASVGDRVTITCRASQDVNTAVAWYQQKPGKAPKLLIYSASFLYSGVPSRFSGSRSGTDFTLTISSLQPEDFATYYCQQYSYYPITFGQGTKVEIKRTGGGSGGGGSGGGASEVQLVESGGGLVQPGGSLRLSCAASGFNLSTHVMHWVRQAPGKGLEWVAEFYPYVGYTYYADSVKGRFTISADTSKNTAYLQMNSLRAEDTAVYYCSRGYRYQYMDVWGQGTLVTVSS

SEQ ID NO: 374 - protein, 240 aa, synthetic construct
DIQMTQSPSSLSASVGDRVTITCRASQDVNTAVAWYQQKPGKAPKLLIYSASFLYSGVPSRFSGSRSGTDFTLTISSLQPEDFATYYCQQSSVEPWTFGQGTKVEIKRTGGGSGGGGSGGGASEVQLVESGGGLVQPGGSLRLSCAASGFNVSYYSIHWVRQAPGKGLEWVAYIYPWNDYTYYADSVKGRFTISADTSKNTAYLQMNSLRAEDTAVYYCSRGSYYSFDYWGQGTLVTVSS

SEQ ID NO: 375 - protein, 238 aa, synthetic construct
DIQMTQSPSSLSASVGDRVTITCRASQDVNTAVAWYQQKPGKAPKLLIYSASFLYSGVPSRFSGSRSGTDFTLTISSLQPEDFATYYCQQSYYSPPTFGQGTKVEIKRTGGGSGGGASEVQLVESGGGLVQPGGSLRLSCAASGFNINNTYIHWVRQAPGKGLEWVASIYPTDGYTRYADSVKGRFTISADTSKNTAYLQMNSLRAEDTAVYYCSRTYYSYYSAMDVWGQGTLVTVSS

SEQ ID NO: 376 - protein, 241 aa, synthetic construct
DIQMTQSPSSLSASVGDRVTITCRASQDVNTAVAWYQQKPGKAPKLLIYSAYFLYSGVPSRFSGSRSGTDFTLTISSLQPEDFATYYCQQIYTSPITFGQGTKVEIKRTGGGSGGGGSGGGASEVQLVESGGGLVQPGGSLRLSCAASGFNFITTGMHWVRQAPGKGLEWVARIGPGSDYTNYADSVKGRFTISADTSKNTAYLQMNSLRAEDTAVYYCSRYYYASALDYWGQGTLVTVSS

SEQ ID NO: 377 - protein, 240 aa, synthetic construct
DIQMTQSPSSLSASVGDRVTITCRASQDVNTAVAWYQQKPGKAPKLLIYSASFLYSGVPSRFSGSRSGTDFTLTISSLQPEDFATYYCQQRAYFPITFGQGTKVEIKRTGGGSGGGGSGGGASEVQLVESGGGLVQPGGSLRLSCAASGFNFSDYGMHWVRQAPGKGLEWVAMLIPASGYTNYADSVKGRFTISADTSKNTAYLQMNSLRAEDTAVYYCSRGWSYYMDYWGQGTLVTVSS

SEQ ID NO: 378 - protein, 241 aa, synthetic construct
DIQMTQSPSSLSASVGDRVTITCRASQDVNTAVAWYQQKPGKAPKLLIYSASFLYSGVPSRFSGSRSGTDFTLTISSLQPEDFATYYCQQQYAYTPITFGQGTKVEIKRTGGGSGGGGSGGGASEVQLVESGGGLVQPGGSLRLSCAASGFNVWSYGIHWVRQAPGKGLEWVAGVTPDGSYTYYADSVKGRFTISADTSKNTAYLQMNSLRAEDTAVYYCSRSYGWAMDYWGQGTLVTVSS

SEQ ID NO: 379 - protein, 241 aa, synthetic construct
DIQMTQSPSSLSASVGDRVTITCRASQDVNTAVAWYQQKPGKAPKLLIYSAYFLYSGVPSRFSGSRSGTDFTLTISSLQPEDFATYYCQQIHYKPLTFGQGTKVEIKRTGGGSGGGGSGGGASEVQLVESGGGLVQPGGSLRLSCAASGFNVAWYSIHWVRQAPGKGLEWVAQVYGGSSYTYYADSVKGRFTISADTSKNTAYLQMNSLRAEDTAVYYCSRDFYSSGMDYWGQGTLVTVSS

SEQ ID NO: 380 - protein, 243 aa, synthetic construct
DIQMTQSPSSLSASVGDRVTITCRASQDVNTAVAWYQQKPGKAPKLLIYSASFLYSGVPSRFSGSRSGTDFTLTISSLQPEDFATYYCQQEWRLPITFGQGTKVEIKRTGGGSGGGGSGGGASEVQLVESGGGLVQPGGSLRLSCAASGFNVYGNQIHWVRQAPGKGLEWVARIYPYSGSTYYADSVKGRFTISADTSKNTAYLQMNSLRAEDTAVYYCSRSAYVAYSYFDYWGQGTLVTVSS

SEQ ID NO: 381-389 - skipped (9 entries)

SEQ ID NO: 390 - protein, 241 aa, synthetic construct
DIQMTQSPSSLSASVGDRVTITCRASQDVNTAVAWYQQKPGKAPKLLIYSASFLYSGVPSRFSGSRSGTDFTLTISSLQPEDFATYYCQQGTSTPFTFGQGTKVEIKRTGGGSGGGGSGGGASEVQLVESGGGLVQPGGSLRLSCAASGFNLSYYGMHWVRQAPGKGLEWVATIYPDSGYTKYADSVKGRFTISADTSKNTAYLQMNSLRAEDTAVYYCSRAYLYYYLAYWGQGTLVTVSS

SEQ ID NO: 391 - protein, 240 aa, synthetic construct
DIQMTQSPSSLSASVGDRVTITCRASQDVNTAVAWYQQKPGKAPKLLIYSASFLYSGVPSRFSGSRSGTDFTLTISSLQPEDFATYYCQQSWRYPMTFGQGTKVEIKRTGGGSGGGGSGGGASEVQLVESGGGLVQPGGSLRLSCAASGFNISRYGMHWVRQAPGKGLEWVAVFYPSSSYTYYADSVKGRFTISADTSKNTAYLQMNSLRAEDTAVYYCSRKYYEAMDYWGQGTLVTVSS

SEQ ID NO: 392 - protein, 240 aa, synthetic construct
DIQMTQSPSSLSASVGDRVTITCRASQDVNTAVAWYQQKPGKAPKLLIYSASFLYSGVPSRFSGSRSGTDFTLTISSLQPEDFATYYCQQSYSYPVTFGHGTKVEIKRTGGGSGGGGSGGGASEVQLVESGGGLVQPGGSLRLSCAASGFNIYSSWMHWVRQAPGKGLEWVAYFQPYSGYTKYADSVKGRFTISADTSKNTAYLQMNSLRAEDTAVYYCSREYTYYFDYWGQGTLVTVSS

SEQ ID NO: 393 - protein, 242 aa, synthetic construct
DIQMTQSPSSLSASVGDRVTITCRASQDVNTAVAWYQQKPGKAPKLLIYSASFLYSGVPSRFSGSRSGTDFTLTISSLQPEDFATYYCQQGWLYSPFTFGQGTKVEIKRTGGGSGGGGSGGGASEVQLVESGGGLVQPGGSLRLSCAASGFNISGYGMHWVRQAPGKGLEWVARVYGGSGYTYYADSVKGRFTISADTSKNTAYLQMNSLRAEDTAVYYCSRAHSSYYVDYWGQGTLVTVSS

SEQ ID NO: 394 - protein, 241 aa, synthetic construct
DIQMTQSPSSLSASVGDRVTITCRASQDVNTAVAWYQQKPGKAPKLLIYSASFLYSGVPSRFSGSRSGTDFTLTISSLQPEDFATYYCQQGYFYYPNTFGQGTKVEIKRTGGGSGGGGSGGGASEVQLVESGGGLVQPGGSLRLSCAASGFNIGYYGMHWVRQAPGKGLEWVATVYPGGGYTSYADSVKGRFTISADTSKNTAYLQMNSLRAEDTAVYYCSRYYYYGFDYWGQGTLVTVSS

SEQ ID NO: 395 - protein, 240 aa, synthetic construct
DIQMTQSPSSLSASVGDRVTITCRASQDVNTAVAWYQQKPGKAPKLLIYSASFLYSGVPSRFSGSRSGTDFTLTISSLQPEDFATYYCQQHYYSPVTFGQGTKVEIKRTGGGSGGGGSGGGASEVQLVESGGGLVQPGGSLRLSCAASGFNIFYQDMHWVRQAPGKGLEWVAMIYPDYDYTYYADSVKGRFTISADTSKNTAYLQMNSLRAEDTAVYYCSRTYSVYMDYWGQGTLVTVSS

SEQ ID NO: 396 - protein, 240 aa, synthetic construct
DIQMTQSPSSLSASVGDRVTITCRASQDVNTAVAWYQQKPGKAPKLLIYSASFLYSGVPSRFSGSRSGTDFTLTISSLQPEDFATYYCQQYAYAPFTFGQGTKVEIKRTGGGSGGGGSGGGASEVQLVESGGGLVQPGGSLRLSCAASGFNVSYSMIHWVRQAPGKGLEWVARVWGDGGVTYYADSVKGRFTISADTSKNTAYLQMNSLRAEDTAVYYCSRGSYYAFDYWGQGTLVTVSS

SEQ ID NO: 397 - protein, 241 aa, synthetic construct
DIQMTQSPSSLSASVGDRVTITCRASQDVNTAVAWYQQKPGKAPKLLIYSASFLYSGVPSRFSGSRSGTDFTLTISSLQPEDFATYYCQQAHMIPITFGQGTKVEIKRTGGGSGGGGSGGGASEVQLVESGGGLVQPGGSLRLSCAASGFNFSFPGMHWVRQAPGKGLEWVAWFVGYDGYTYYADSVKGRFTISADTSKNTAYLQMNSLRAEDTAVYYCSRDYYSFSMDYWGQGTLVTVSS

SEQ ID NO: 398 - protein, 240 aa, synthetic construct
DIQMTQSPSSLSASVGDRVTITCRASQDVNTAVAWYQQKPGKAPKLLIYSASFLYSGVPSRFSGSRSGTDFTLTISSLQPEDFATYYCQQSVYDPITFGQGTKVEIKRTGGGSGGGGSGGGASEVQLVESGGGLVQPGGSLRLSCAASGFNISGSWIHWVRQAPGKGLEWVAWLYPDSDYTYYADSVKGRFTISADTSKNTAYLQMNSLRAEDTAVYYCSRAHTYAFDYWGQGTLVTVSS

SEQ ID NO: 399 - protein, 249 aa, synthetic construct
DIQMTQSPSSLSASVGDRVTITCRASQDVNTAVAWYQQKPGKAPKLLIYSASFLYSGVPSRFSGSRSGTDFTLTISSLQPEDFATYYCQQSYTSPLTFGQGTKVEIKRTGGGSGGGGSGGGASEVQLVESGGGLVQPGGSLRLSCAASGFNIYYGVMHWVRQAPGKGLEWVAMIYPDSSWTYYADSVKGRFTISADTSKNTAYLQMNSLRAEDTAVYYCSRDQDFHYMNYYLSYALDYWGQGTLVTVSS

SEQ ID NO: 400 - protein, 240 aa, synthetic construct
DIQMTQSPSSLSASVGDRVTITCRASQDVNTAVAWYQQKPGKAPKLLIYSASFLYSGVPSRFSGSRSGTDFTLTISSLQPEDFATYYCQQGQYSPFTFGQGTKVEIKRTGGGSGGGGSGGGASEVQLVESGGGLVQPGGSLRLSCAASGFNVSYEYMHWVRQAPGKGLEWVAEIYGGSDNTYYADSVKGRFTISADTSKNTAYLQMNSLRAEDTAVYYCSRPLGSYFDYWGQGTLVTVSS

SEQ ID NO: 401 - protein, 241 aa, synthetic construct
DIQMTQSPSSLSASVGDRVTITCRASQDVNTAVAWYQQKPGKAPKLLIYSASFLYSGVPSRFSGSRSGTDFTLTISSLQPEDFATYYCQQYWYLPTTFGQGTKVEIKRTGGGSGGGGSGGGASEVQLVESGGGLVQPGGSLRLSCAASGFNISWYDIHWVRQAPGKGLEWVADIEPSVGYTYYADSVKGRFTISADTSKNTAYLQMNSLRAEDTAVYYCSRSYPYYYFDYWGQGTLVTVSS

SEQ ID NO: 402 - protein, 8 aa, synthetic construct
GFNLSYYG

SEQ ID NO: 403 - protein, 10 aa, synthetic construct
ELAGIGILTV

SEQ ID NO: 404 - protein, 244 aa, synthetic construct
DIQMTQSPSSLSASVGDRVTITCRASQDIRNYLNWYQQKPGKAPKLLIYYTSRLESGVPSRFSGSGSGTDYTLTISSLQPEDFATYYCQQGNTLPWTFGQGTKVEIKGGGGSGGGGSGGGGSEVQLVESGGGLVQPGGSLRLSCAASGYSFTGYTMNWVRQAPGKGLEWVALINPYKGVSTYNQKFKDRFTISVDKSKNTAYLQMNSLRAEDTAVYYCARSGYYGDSDWYFDVWGQGTLVTVSS

SEQ ID NO: 405 - protein, 244 aa, synthetic construct
DIQMTQTTSSLSASLGDRVTISCRASQDIRNYLNWYQQKPDGTVKLLIYYTSRLHSGVPSKFSGSGSGTDYSLTISNLEQEDIATYFCQQGNTLPWTFAGGTKLEIKGGGGSGGGGSGGGGSEVQLQQSGPELVKPGASMKISCKASGYSFTGYTMNWVKQSHGKNLEWMGLINPYKGVSTYNQKFKDKATLTVDKSSSTAYMELLSLTSEDSAVYYCARSGYYGDSDWYFDVWGAGTTVTVSS

SEQ ID NO: 406 - protein, 240 aa, synthetic construct
DIVLTQSPATLSLSPGERATLSCRASQSVSYMNWYQQKPGKAPKRWIYDTSKVASGVPARFSGSGSGTDYSLTINSLEAEDAATYYCQQWSSNPLTFGGGTKVEIKGGGGSGGGGSGGGGSDVQLVQSGAEVKKPGASVKVSCKASGYTFTRYTMHWVRQAPGQGLEWIGYINPSRGYTNYADSVKGRFTITTDKSTSTAYMELSSLRSEDTATYYCARYYDDHYCLDYWGQGTTVTVSS

SEQ ID NO: 407 - protein, 249 aa, synthetic construct
QAVVTQEPSLTVSPGGTVTLTCRSSTGAVTTSNYANWVQQKPGQAPRGLIGGTNKRAPWTPARFSGSLLGGKAALTITGAQAEDEADYYCALWYSNLWVFGGGTKLTVLGGGGSGGGGSGGGGSEVQLVESGGGLVQPGGSLRLSCAASGFTFNTYAMNWVRQAPGKGLEWVARIRSKYNNYATYYADSVKDRFTISRDDSKNSLYLQMNSLKTEDTAVYYCVRHGNFGNSYVSWFAYWGQGTLVTVSS

SEQ ID NO: 408 - protein, 240 aa, synthetic construct
DIQLTQSPAIMSASPGEKVTMTCRASSSVSYMNWYQQKSGTSPKRWIYDTSKVASGVPYRFSGSGSGTSYSLTISSMEAEDAATYYCQQWSSNPLTFGAGTKLELKGGGGSGGGGSGGGGSDIKLQQSGAELARPGASVKMSCKTSGYTFTRYTMHWVKQRPGQGLEWIGYINPSRGYTNYNQKFKDKATLTTDKSSSTAYMQLSSLTSEDSAVYYCARYYDDHYCLDYWGQGTTLTVSS

SEQ ID NO: 409 - protein, 240 aa, synthetic construct
QIVLTQSPAIMSASPGEKVTMTCSASSSVSYMNWYQQKSGTSPKRWIYDTSKLASGVPAHFRGSGSGTSYSLTISGMEAEDAATYYCQQWSSNPFTFGSGTKLEINGGGGSGGGGSGGGGSQVQLQQSGAELARPGASVKMSCKASGYTFTRYTMHWVKQRPGQGLEWIGYINPSRGYTNYNQKFKDKATLTTDKSSSTAYMQLSSLTSEDSAVYYCARYYDDHYCLDYWGQGTTLTVSS

SEQ ID NO: 410 - protein, 249 aa, synthetic construct
QTVVTQEPSLTVSPGGTVTLTCGSSTGAVTSGNYPNWVQQKPGQAPRGLIGGTKFLAPGTPARFSGSLLGGKAALTLSGVQPEDEAEYYCVLWYSNRWVFGGGTKLTVLGGGGSGGGGSGGGGSEVQLVESGGGLVQPGGSLKLSCAASGFTFNKYAMNWVRQAPGKGLEWVARIRSKYNNYATYYADSVKDRFTISRDDSKNTAYLQMNNLKTEDTAVYYCVRHGNFGNSYISYWAYWGQGTLVTVSS

SEQ ID NO: 411 - protein, 241 aa, synthetic construct
EIVLTQSPATLSLSPGERATLSCRASQSVSSYLAWYQQKPGQAPRLLIYDASNRATGIPARFSGSGSGTDFTLTISSLEPEDFAVYYCQQRSNWPPLTFGGGTKVEIKGGGGSGGGGSGGGGSQVQLVESGGGVVQPGRSLRLSCAASGFKFSGYGMHWVRQAPGKGLEWVAVIWYDGSKKYYVDSVKGRFTISRDNSKNTLYLQMNSLRAEDTAVYYCARQMGYWHFDLWGRGTLVTVSS

SEQ ID NO: 412 - protein, 241 aa, synthetic construct
EIVLTQSPRTLSLSPGERATLSCRASQSVSSSYLAWYQQKPGQAPRLLIYGASSRATGIPDRFSGSGSGTDFTLTISRLDPEDFAVYYCQQYGSSPITFGQGTRLEIKGGGGSGGGGSGGGGSQVQLVESGGGVVQPGRSLRLSCAASGFTFRSYGMHWVRQAPGKGLEWVAIIWYDGSKKNYADSVKGRFTISRDNSKNTLYLQMNSLRAEDTAVYYCARGTGYNWFDPWGQGTLVTVSS

SEQ ID NO: 413 - protein, 239 aa, synthetic construct
DILMTQSPSSLSASVGDRVTITCRASQGISSALAWYQQKPGKAPKLLIYYASSLQSGVPSRFSGSGSGTDYTLTISSLQPEDFATYYCQQYYSTLTFGGGTKVEIKGGGGSGGGGSGGGGSQVQLVESGGGVVQPGRSLRLSCAASGFTFRSYGMHWVRQAPGKGLEWVAIIWYDGSKKNYADSVKGRFTISRDNSKNTLYLQMNSLRAEDTAVYYCARGTGYNWFDPWGQGTLVTVSS

SEQ ID NO: 414 - protein, 241 aa, synthetic construct
EIVLTQSPATLSLSPGERATLSCRASQSVSSYLAWYQQKPGQAPRLLIYDASNRATGIPARFSGSGSGTDFTLTISSLEPEDFAVYYCQQRSNWPPLTFGGGTKVEIKGGGGSGGGGSGGGGSQVQLVQSGGGVVQSGRSLRLSCAASGFKFSGYGMHWVRQAPGKGLEWVAVIWYDGSKKYYVDSVKGRFTISRDNSKNTLYLQMNSLRGEDTAVYYCARQMGYWHFDLWGRGTLVTVSS

SEQ ID NO: 415 - protein, 240 aa, synthetic construct
EIVLTQSPATLSLSPGERATLSCRASQSVSSYLAWYQQKPGQAPRLLIYDASNRATGIPARFSGSGSGTDFTLTISSLEPEDFAVYYCQQRSNWPWTFGQGTKVEIKGGGGSGGGGSGGGGSQVQLVQSGGGVVQPGRSLRLSCVASGFTFSSYGMHWVRQAPGKGLEWVAAIWYNGRKQDYADSVKGRFTISRDNSKNTLYLQMNSLRAEDTAVYYCTRGTGYNWFDPWGQGTLVTVSS

SEQ ID NO: 416 - protein, 240 aa, synthetic construct
AIQLTQSPSSLSASVGDRVTITCRASQGISSALAWYQQKPGKAPKLLIYDASSLESGVPSRFSGSGSGTDFTLTISSLQPEDFATYYCQQFNSYPITFGQGTRLEIKGGGGSGGGGSGGGGSQVQLVQSGGGVVQPGRSLRLSCVASGFTFSSYGMHWVRQAPGKGLEWVAAIWYNGRKQDYADSVKGRFTISRDNSKNTLYLQMNSLRAEDTAVYYCTRGTGYNWFDPWGQGTLVTVSS

SEQ ID NO: 417 - protein, 241 aa, synthetic construct
QIVLSQSPAILSASPGEKVTMTCRASSSVSYMHWYQQKPGSSPKPWIYATSNLASGVPARFSGSGSGTSYSLTISRVEAEDAATYYCQQWSSNPPTFGGGTKLETKRGGGGSGGGGSGGGGSQVQLQQSGAELARPGASVKMSCKASGYTFTSYTMHWVKQRPGQGLEWIGYINPSSGYTKYNQKFKDKATLTADKSSSTAYMQLSSLTSEDSAVYYCARWQDYDVYFDYWGQGTTLTVSS

SEQ ID NO: 418 - protein, 10 aa, synthetic construct
SPGAANKRPI

SEQ ID NO: 419 - protein, 9 aa, synthetic construct
VVGACGVGK

SEQ ID NO: 420 - protein, 9 aa, synthetic construct
VVGADGVGK